European Patent Application EP 4 696 717 A1, published February 18, 2026. Title: NEW CHIMERIC OPSIN GPCR PROTEIN FOR TREATING RETINAL NEURODEGENERATIVE DISEASES. Applicant: SUZHOU UGENEX THERAPEUTICS CO., LTD. Application US. The sequence listing filed with the application follows.

SEQUENCE LISTING (9 sequences)

SEQ ID NO: 1 - protein, 412 aa, synthetic construct
MAQQWSLQRLAGRHPQDSYEDSTQSSIFTYTNSNSTRGPFEGPNYHIAPRWVYHLTSVWMIFVVIASVFTNGLVLAATMKFKKLRHPLNWILVNLAVADLAETVIASTISVVNQVYGYFVLGHPMCVLEGYTVSLCGITGLWSLAIISWERIYRIFEQGKRSVSAPRFISPASQVGIAFSWIWAAVWTAPPIFGWSRYWPHGLKTSCGPDVFSGSSYPGVQSYMIVLMVTCCITPLSIIVLCYLQVWLKTRGVPETFNEAKMVVVMVLAFCFCWGPYAFFACFAAANPGYPFHPLMAALPAFFAKSATIYNPVIYVFMNRQPEQNVPKRKRSLKAVVTAATMSNKFTQKGNFRPNGEAKSELCENLEAPALATKQTYVTYTNHAIRSRFVKKDGHCNVQFINVTETSQVAPA

SEQ ID NO: 2 - DNA, 1236 bp, synthetic construct
  source 1..1236: mol_type = other DNA
atggctcagcaatggagtttgcagagactggctggtaggcatcctcaggatagctacgaggacagcactcagtctagtatttttacctacacaaactccaacagcacaagaggccctttcgagggcccgaattaccacatagcgcccaggtgggtgtaccatcttactagcgtttggatgatctttgtggtgatcgcgtccgtgttcactaacgggctggtgctggctgctactatgaagttcaaaaagctgcggcatccactgaactggatactggttaatctcgccgtggccgacctggctgagacagttatcgctagcaccatttctgttgtgaatcaggtctacgggtattttgtcctcgggcatccaatgtgtgtgctggaaggctatacggtaagcctttgcggaatcaccggcctgtggagcctcgcaataatctcctgggaacgaatttaccggatcttcgagcaagggaaacgatctgtgagtgcccctaggttcatcagtcccgccagccaggttggaattgcctttagctggatttgggcagctgtatggacagcaccaccaatttttggatggagcagatattggccccacgggctcaaaaccagctgtggccctgatgtgttttctggatcatcctaccctggtgttcagagttatatgattgtgttgatggttacatgctgcatcacaccgctgtcaatcatcgtgctttgctatctccaggtctggctcaagactaggggggtccctgaaacctttaatgaggccaaaatggtcgtcgtgatggtgctggctttctgtttctgctgggggccctatgctttctttgcatgcttcgcagccgccaatcctggctacccatttcatccactgatggctgctttgccagcgtttttcgcgaaaagtgctactatctacaatcccgtcatctacgtgtttatgaacagacaacccgaacagaacgtcccaaagagaaagaggtcactgaaggctgtggttaccgccgccactatgtcaaacaagtttacccagaagggtaattttcgccccaatggagaggcaaagtccgagctttgtgagaatttggaggcgcccgccctggctaccaaacaaacatatgtgacatacaccaatcacgccatcagaagccgctttgtgaagaaagatggtcattgcaatgtgcagtttattaatgtgaccgagacctcacaggttgccccagcc

SEQ ID NO: 3 - protein, 385 aa, synthetic construct
MAQQWSLQRLAGRHPQDSYEDSTQSSIFTYTNSNSTRGPFEGPNYHIAPRWVYHLTSVWMIFVVIASVFTNGLVLAATMKFKKLRHPLNWILVNLAVADLAETVIASTISVVNQVYGYFVLGHPMCVLEGYTVSLCGITGLWSLAIISWERIYRIFEQGKRSVSAPRFISPASQVGIAFSWIWAAVWTAPPIFGWSRYWPHGLKTSCGPDVFSGSSYPGVQSYMIVLMVTCCITPLSIIVLCYLQVWLKTRGVPETFNEAKMVVVMVLAFCFCWGPYAFFACFAAANPGYPFHPLMAALPAFFAKSATIYNPVIYVFMNRQPEQNVPKRKRSLKAVVTAATMSNKFTQKGNFRPNGEAKSELCENLEAPALATKQTYVTYTNHAI

SEQ ID NO: 4 - DNA, 1155 bp, synthetic construct
  source 1..1155: mol_type = other DNA
atggctcagcaatggagtttgcagagactggctggtaggcatcctcaggatagctacgaggacagcactcagtctagtatttttacctacacaaactccaacagcacaagaggccctttcgagggcccgaattaccacatagcgcccaggtgggtgtaccatcttactagcgtttggatgatctttgtggtgatcgcgtccgtgttcactaacgggctggtgctggctgctactatgaagttcaaaaagctgcggcatccactgaactggatactggttaatctcgccgtggccgacctggctgagacagttatcgctagcaccatttctgttgtgaatcaggtctacgggtattttgtcctcgggcatccaatgtgtgtgctggaaggctatacggtaagcctttgcggaatcaccggcctgtggagcctcgcaataatctcctgggaacgaatttaccggatcttcgagcaagggaaacgatctgtgagtgcccctaggttcatcagtcccgccagccaggttggaattgcctttagctggatttgggcagctgtatggacagcaccaccaatttttggatggagcagatattggccccacgggctcaaaaccagctgtggccctgatgtgttttctggatcatcctaccctggtgttcagagttatatgattgtgttgatggttacatgctgcatcacaccgctgtcaatcatcgtgctttgctatctccaggtctggctcaagactaggggggtccctgaaacctttaatgaggccaaaatggtcgtcgtgatggtgctggctttctgtttctgctgggggccctatgctttctttgcatgcttcgcagccgccaatcctggctacccatttcatccactgatggctgctttgccagcgtttttcgcgaaaagtgctactatctacaatcccgtcatctacgtgtttatgaacagacaacccgaacagaacgtcccaaagagaaagaggtcactgaaggctgtggttaccgccgccactatgtcaaacaagtttacccagaagggtaattttcgccccaatggagaggcaaagtccgagctttgtgagaatttggaggcgcccgccctggctaccaaacaaacatatgtgacatacaccaatcacgccatc

SEQ ID NO: 5 - protein, 23 aa, synthetic construct
IYRIFEQGKRSVSAPRFISPASQ

SEQ ID NO: 6 - protein, 13 aa, synthetic construct
KTRGVPETFNEAK

SEQ ID NO: 7 - protein, 64 aa, synthetic construct
PEQNVPKRKRSLKAVVTAATMSNKFTQKGNFRPNGEAKSELCENLEAPALATKQTYVTYTNHAI

SEQ ID NO: 8 - protein, 18 aa, synthetic construct
RSRFVKKDGHCNVQFINV

SEQ ID NO: 9 - protein, 9 aa, synthetic construct
TETSQVAPA